European Patent Application EP 4 353 749 A1, published April 17, 2024. Title: ANTI-MASP-2 ANTIBODY AND USE THEREOF. Applicant: SHANGHAI JEMINCARE PHARMACEUTICAL CO., LTD; JIANGXI JEMINCARE GROUP CO., LTD. The sequence listing filed with the application follows.

SEQUENCE LISTING (77 sequences)

SEQ ID NO: 1 - protein, 433 aa, Artificial Sequence
  hMASP2-D456
MASMTGWKIHYTSTAHACPYPMAPPNGHVSPVQAKYILKDSFSIFCETGYELLQGHLPLKSFTAVCQKDGSWDRPMPACSIVDCGPPDDLPSGRVEYITGPGVTTYKAVIQYSCEETFYTMKVNDGKYVCEADGFWTSSKGEKSLPVCEPVCGLSARTTGGRIYGGQKAKPGDFPWQVLILGGTTAAGALLYDNWVLTAAHAVYEQKHDASALDIRMGTLKRLSPHYTQAWSEAVFIHEGYTHDAGFDNDIALIKLNNKVVINSNITPICLPRKEAESFMRTDDIGTASGWGLTQRGFLARNLMYVDIPIVDHQKCTAAYEKPPYPRGSVTANMLCAGLESGGKDSCRGDSGGALVFLDSETERWFVGGIVSWGSMNCGEAGQYGVYTKVINYIPWIENIISDFGGGGSGGGGSAKFVAAWTLKAAAHHHHHH

SEQ ID NO: 2 - protein, 432 aa, Artificial Sequence
  hMASP2A-D456
MASMTGWKIHYTSTAHACPYPMAPPNGHVSPVQAKYILKDSFSIFCETGYELLQGHLPLKSFTAVCQKDGSWDRPMPACSIVDCGPPDDLPSGRVEYITGPGVTTYKAVIQYSCEETFYTMKVNDGKYVCEADGFWTSSKGEKSLPVCEPVCGLSARTTGGRIYGGQKAKPGDFPWQVLILGGTTAAGALLYDNWVLTAAHAVYEQKHDASALDIRMGTLKRLSPHYTQAWSEAVFIHEGYTHDAGFDNDIALIKLNNKVVINSNITPICLPRKEAESFMRTDDIGTASGWGLTQRGFLARNLMYVDIPIVDHQKCTAAYEKPPYPRGSVTANMLCAGLESGGKDSCRGDAGGALVFLDSETERWFVGGIVSWGSMNCGEAGQYGVYTKVINYIPWIENIISDFGGGGSGGGGSAKFVAAWTLKAAAHHHHH

SEQ ID NO: 3 - protein, 432 aa, Artificial Sequence
  mMASP2-D456
MASMTGWKIHYTSTARPCPDPTAPPNGSISPVQAIYVLKDRFSVFCKTGFELLQGSVPLKSFTAVCQKDGSWDRPMPECSIIDCGPPDDLPNGHVDYITGPEVTTYKAVIQYSCEETFYTMSSNGKYVCEADGFWTSSKGEKLPPVCEPVCGLSTHTIGGRIVGGQPAKPGDFPWQVLLLGQTTAAAGALIHDNWVLTAAHAVYEKRMAASSLNIRMGILKRLSPHYTQAWPEEIFIHEGYTHGAGFDNDIALIKLKNKVTINGSIMPVCLPRKEAASLMRTDFTGTVAGWGLTQKGLLARNLMFVDIPIADHQKCTAVYEKLYPGVRVSANMLCAGLETGGKDSCRGDSGGALVFLDNETQRWFVGGIVSWGSINCGAADQYGVYTKVINYIPWIENIISNFGGGGSGGGGSAKFVAAWTLKAAAHHHHHH

SEQ ID NO: 4 - protein, 433 aa, Artificial Sequence
  cMASP2-D456
MASMTGWKIHYTSTAQPCPYPMAPPNGHLSPVQAKYILKDSFSIFCEPGYELLQGHLPLKSFAAVCQKDGSWDQPMPSCSIVDCGPPDDLPSGRVEYITGPEVTTYKAVIQYSCEETFYTMKVNDGKYVCEADGFWTSSKGERSPPVCEPVCGLSARTTGGRIYGGQKAKPGDFPWQVLILGGSTAAGALLYDNWVLTAAHAIYEQKHDASSLDIRLGALKRLSPHYTQAWAEAVFIHEGYTHDAGFDNDIALIKLNNKVVINSNITPICLPRKEAESFMRTDDIGTASGWGLTQRGLLARNLMYVDIPIVDHQKCTAAYEKPPYSGGSVTANMLCAGLESGGKDSCRGDSGGALVFLDNETQRWFVGGIVSWGSMNCGEAGQYGVYTKVINYIPWIKNIISNFGGGGSGGGGSAKFVAAWTLKAAAHHHHHH

SEQ ID NO: 5 - protein, 107 aa, Artificial Sequence
  Light chain variable region of 50A6
NIVLTQSPATLSVTPGESVSLSCRASQSVSTSIHWYQQRSNESPRLLIKYASRSISGIPSRFSGSGSGTDFTLSINRVESEDFSIYYCQQSYSSLYTFGAGTKLELR

SEQ ID NO: 6 - protein, 23 aa, Artificial Sequence
  50A6 L-FR1
NIVLTQSPATLSVTPGESVSLSC

SEQ ID NO: 7 - protein, 11 aa, Artificial Sequence
  50A6 LCDR1, JYB1931A63 LCDR1
RASQSVSTSIH

SEQ ID NO: 8 - protein, 15 aa, Artificial Sequence
  50A6 L-FR2
WYQQRSNESPRLLIK

SEQ ID NO: 9 - protein, 7 aa, Artificial Sequence
  50A6 LCDR2, JYB1931A63 LCDR2
YASRSIS

SEQ ID NO: 10 - protein, 32 aa, Artificial Sequence
  50A6 L-FR3
GIPSRFSGSGSGTDFTLSINRVESEDFSIYYC

SEQ ID NO: 11 - protein, 9 aa, Artificial Sequence
  50A6 LCDR3, JYB1931A63 LCDR3
QQSYSSLYT

SEQ ID NO: 12 - protein, 10 aa, Artificial Sequence
  50A6 L-FR4
FGAGTKLELR

SEQ ID NO: 13 - protein, 125 aa, Artificial Sequence
  Heavy chain variable region of 50A6
EVQLVESGGGLVQPGRSLSLSCAASGFTFNDYNMAWVRQTPKKGLEWVATILFDGSRTYYRDSVKGRFTISRENAKSTLYLQMDSLRSEDTATYYCSTESPYYSEGYYQGYFDYWGQGVMVTVSS

SEQ ID NO: 14 - protein, 25 aa, Artificial Sequence
  50A6 H-FR1
EVQLVESGGGLVQPGRSLSLSCAAS

SEQ ID NO: 15 - protein, 7 aa, Artificial Sequence
  50A6 HCDR1, JYB1931A63 HCDR1
GFTFNDY

SEQ ID NO: 16 - protein, 19 aa, Artificial Sequence
  50A6 H-FR2
NMAWVRQTPKKGLEWVATI

SEQ ID NO: 17 - protein, 6 aa, Artificial Sequence
  50A6 HCDR2, JYB1931A63 HCDR2
LFDGSR

SEQ ID NO: 18 - protein, 41 aa, Artificial Sequence
  50A6 H-FR3
TYYRDSVKGRFTISRENAKSTLYLQMDSLRSEDTATYYCST

SEQ ID NO: 19 - protein, 16 aa, Artificial Sequence
  50A6 HCDR3;JYB1931A63 HCDR3
ESPYYSEGYYQGYFDY

SEQ ID NO: 20 - protein, 11 aa, Artificial Sequence
  50A6 H-FR4
WGQGVMVTVSS

SEQ ID NO: 21 - protein, 107 aa, Artificial Sequence
  Light chain variable region of JYB1931A63
EIVLTQSPATLSLSPGERATLSCRASQSVSTSIHWYQQKPGQAPRLLIKYASRSISGIPARFSGSGSGTDFTLTISSLEPEDFAVYYCQQSYSSLYTFGQGTKLEIK

SEQ ID NO: 22 - protein, 23 aa, Artificial Sequence
  JYB1931A63 L-FR1
EIVLTQSPATLSLSPGERATLSC

SEQ ID NO: 23 - protein, 15 aa, Artificial Sequence
  JYB1931A63 L-FR2
WYQQKPGQAPRLLIK

SEQ ID NO: 24 - protein, 32 aa, Artificial Sequence
  JYB1931A63 L-FR3
GIPARFSGSGSGTDFTLTISSLEPEDFAVYYC

SEQ ID NO: 25 - protein, 10 aa, Artificial Sequence
  JYB1931A63 L-FR4
FGQGTKLEIK

SEQ ID NO: 26 - protein, 125 aa, Artificial Sequence
  Heavy chain variable region of JYB1931A63
EVQLVESGGGLVQPGGSLRLSCAASGFTFNDYNMAWVRQAPGKGLEWVATILFDGSRTYYRDSVKGRFTISRDNAKNSLYLQMNSLRAEDTAVYYCSTESPYYSEGYYQGYFDYWGQGTLVTVSS

SEQ ID NO: 27 - protein, 25 aa, Artificial Sequence [sequence omitted]

SEQ ID NO: 28 - protein, 19 aa, Artificial Sequence
  JYB1931A63 H-FR2
NMAWVRQAPGKGLEWVATI

SEQ ID NO: 29 - protein, 41 aa, Artificial Sequence
  JYB1931A63 H-FR3
TYYRDSVKGRFTISRDNAKNSLYLQMNSLRAEDTAVYYCST

SEQ ID NO: 30 - protein, 11 aa, Artificial Sequence
  JYB1931A63 H-FR4;JYB1931A13 H-FR4
WGQGTLVTVSS

SEQ ID NO: 31 - protein, 107 aa, Artificial Sequence
  Light chain variable region of 47A1
DIVMTQSQKFMSTSVGDRVSVTCKASQNVGSNVAWFQQKPGQSPKPLIYSASYRYSGVPDRFTGSGSGTDFTLTISNVQSEDLAEYFCHQYNTYPLTFGAGTKLELN

SEQ ID NO: 32 - protein, 23 aa, Artificial Sequence
  47A1 L-FR1
DIVMTQSQKFMSTSVGDRVSVTC

SEQ ID NO: 33 - protein, 11 aa, Artificial Sequence
  47A1 LCDR1;JYB1931A13 LCDR1
KASQNVGSNVA

SEQ ID NO: 34 - protein, 15 aa, Artificial Sequence
  47A1 L-FR2
WFQQKPGQSPKPLIY

SEQ ID NO: 35 - protein, 7 aa, Artificial Sequence
  47A1 LCDR2;JYB1931A13 LCDR2
SASYRYS

SEQ ID NO: 36 - protein, 32 aa, Artificial Sequence
  47A1 L-FR3
GVPDRFTGSGSGTDFTLTISNVQSEDLAEYFC

SEQ ID NO: 37 - protein, 9 aa, Artificial Sequence
  47A1 LCDR3;JYB1931A13 LCDR3
HQYNTYPLT

SEQ ID NO: 38 - protein, 10 aa, Artificial Sequence
  47A1 L-FR4
FGAGTKLELN

SEQ ID NO: 39 - protein, 114 aa, Artificial Sequence
  Heavy chain variable region of  47A1
DVQLQESGPGLVKPSQSLSLTCTVTGYSITSDYAWNWIRQFPGNKLEWMGYISYSGRTSYNPSLKSRISITRNTSTNQFFLQLNSVTTEDTATYFCARYWGDYWGQGTTLTVSS

SEQ ID NO: 40 - protein, 25 aa, Artificial Sequence
  47A1 H-FR1
DVQLQESGPGLVKPSQSLSLTCTVT

SEQ ID NO: 41 - protein, 8 aa, Artificial Sequence
  47A1 HCDR1;JYB1931A13 HCDR1
GYSITSDY

SEQ ID NO: 42 - protein, 19 aa, Artificial Sequence
  47A1 H-FR2
AWNWIRQFPGNKLEWMGYI

SEQ ID NO: 43 - protein, 5 aa, Artificial Sequence
  47A1 HCDR2;JYB1931A13 HCDR2
SYSGR

SEQ ID NO: 44 - protein, 41 aa, Artificial Sequence
  47A1 H-FR3
TSYNPSLKSRISITRNTSTNQFFLQLNSVTTEDTATYFCAR

SEQ ID NO: 45 - protein, 5 aa, Artificial Sequence
  47A1 HCDR3;JYB1931A13 HCDR3
YWGDY

SEQ ID NO: 46 - protein, 11 aa, Artificial Sequence
  47A1 H-FR4
WGQGTTLTVSS

SEQ ID NO: 47 - protein, 107 aa, Artificial Sequence
  Light chain variable region of JYB1931A13
DIQMTQSPSSLSASVGDRVTITCKASQNVGSNVAWFQQKPGKAPKPLIYSASYRYSGVPSRFSGSGSGTDFTLTISSLQPEDFATYFCHQYNTYPLTFGGGTKVEIK

SEQ ID NO: 48 - protein, 23 aa, Artificial Sequence
  JYB1931A13 L-FR1
DIQMTQSPSSLSASVGDRVTITC

SEQ ID NO: 49 - protein, 15 aa, Artificial Sequence
  JYB1931A13 L-FR2
WFQQKPGKAPKPLIY

SEQ ID NO: 50 - protein, 32 aa, Artificial Sequence
  JYB1931A13 L-FR3
GVPSRFSGSGSGTDFTLTISSLQPEDFATYFC

SEQ ID NO: 51 - protein, 10 aa, Artificial Sequence
  JYB1931A13 L-FR4
FGGGTKVEIK

SEQ ID NO: 52 - protein, 114 aa, Artificial Sequence
  Heavy chain variable region of JYB1931A13
QVQLQESGPGLVKPSQTLSLTCTVSGYSITSDYAWNWIRQPPGKGLEWIGYISYSGRTSYNPSLKSRVTISRDTSKNQFSLKLSSVTAADTAVYYCARYWGDYWGQGTLVTVSS

SEQ ID NO: 53 - protein, 25 aa, Artificial Sequence
  JYB1931A13 H-FR1
QVQLQESGPGLVKPSQTLSLTCTVS

SEQ ID NO: 54 - protein, 19 aa, Artificial Sequence
  JYB1931A13 H-FR2
AWNWIRQPPGKGLEWIGYI

SEQ ID NO: 55 - protein, 41 aa, Artificial Sequence
  JYB1931A13 H-FR3
TSYNPSLKSRVTISRDTSKNQFSLKLSSVTAADTAVYYCAR

SEQ ID NO: 56 - protein, 327 aa, Artificial Sequence
  Heavy chain variable region of JYB1931A63;heavy chain variable region of JYB1931A13
ASTKGPSVFPLAPCSRSTSESTAALGCLVKDYFPEPVTVSWNSGALTSGVHTFPAVLQSSGLYSLSSVVTVPSSSLGTKTYTCNVDHKPSNTKVDKRVESKYGPPCPPCPAPEFLGGPSVFLFPPKPKDTLMISRTPEVTCVVVDVSQEDPEVQFNWYVDGVEVHNAKTKPREEQFNSTYRVVSVLTVLHQDWLNGKEYKCKVSNKGLPSSIEKTISKAKGQPREPQVYTLPPSQEEMTKNQVSLTCLVKGFYPSDIAVEWESNGQPENNYKTTPPVLDSDGSFFLYSRLTVDKSRWQEGNVFSCSVMHEALHNHYTQKSLSLSLGK

SEQ ID NO: 57 - protein, 107 aa, Artificial Sequence [sequence omitted]

SEQ ID NO: 58 - protein, 23 aa, Artificial Sequence
  general formula 1 of  L-FR1
  misc_feature (1)..(1): Xaa = Glu or Asn
  misc_feature (13)..(13): Xaa = Leu or Val
  misc_feature (14)..(14): Xaa = Ser or Thr
  misc_feature (18)..(18): Xaa = Arg or Ser
  misc_feature (19)..(19): Xaa = Ala or Val
  misc_feature (20)..(20): Xaa = Ser or Thr
XIVLTQSPATLSXXPGEXXXLSC

SEQ ID NO: 59 - protein, 15 aa, Artificial Sequence
  general formula 1 of  L-FR2
  misc_feature (5)..(5): Xaa = Lys or Arg
  misc_feature (6)..(6): Xaa = Pro or Ser
  misc_feature (7)..(7): Xaa = Gly or Asn
  misc_feature (8)..(8): Xaa = Glu or Gln
  misc_feature (9)..(9): Xaa = Ala or Ser
WYQQXXXXXPRLLIK

SEQ ID NO: 60 - protein, 32 aa, Artificial Sequence
  general formula 1 of L-FR3
  misc_feature (4)..(4): Xaa = Ala or Ser
  misc_feature (18)..(18): Xaa = Ser or Thr
  misc_feature (20)..(20): Xaa = Asn or Ser
  misc_feature (21)..(21): Xaa = Arg or Ser
  misc_feature (22)..(22): Xaa = Leu or Val
  misc_feature (24)..(24): Xaa = Pro or Ser
  misc_feature (28)..(28): Xaa = Ala or Ser
  misc_feature (29)..(29): Xaa = Ile or Val
GIPXRFSGSGSGTDFTLXIXXXEXEDFXXYYC

SEQ ID NO: 61 - protein, 10 aa, Artificial Sequence
  general formula 1 of L-FR4
  misc_feature (3)..(3): Xaa = Ala or Gln
  misc_feature (9)..(9): Xaa = Ile or Leu
  misc_feature (10)..(10): Xaa = Lys or Arg
FGXGTKLEXX

SEQ ID NO: 62 - protein, 25 aa, Artificial Sequence
  general formula 1 of H-FR1
  misc_feature (16)..(16): Xaa = Gly or Arg
  misc_feature (19)..(19): Xaa = Arg or Ser
EVQLVESGGGLVQPGXSLXLSCAAS

SEQ ID NO: 63 - protein, 19 aa, Artificial Sequence
  general formula 1 of H-FR2
  misc_feature (8)..(8): Xaa = Ala or Thr
  misc_feature (10)..(10): Xaa = Gly or Lys
NMAWVRQXPXKGLEWVATI

SEQ ID NO: 64 - protein, 41 aa, Artificial Sequence
  general formula 1 of H-FR3
  misc_feature (16)..(16): Xaa = Asp or Glu
  misc_feature (20)..(20): Xaa = Asn or Ser
  misc_feature (21)..(21): Xaa = Ser or Thr
  misc_feature (27)..(27): Xaa = Asp or Asn
  misc_feature (31)..(31): Xaa = Ala or Ser
  misc_feature (36)..(36): Xaa = Thr or Val
TYYRDSVKGRFTISRXNAKXXLYLQMXSLRXEDTAXYYCST

SEQ ID NO: 65 - protein, 11 aa, Artificial Sequence
  general formula 1 of H-FR4
  misc_feature (5)..(5): Xaa = Thr or Val
  misc_feature (6)..(6): Xaa = Leu or Met
WGQGXXVTVSS

SEQ ID NO: 66 - protein, 107 aa, Artificial Sequence
  general formula 1 of VL
  misc_feature (1)..(1): Xaa = Glu or Asn
  misc_feature (13)..(13): Xaa = Leu or Val
  misc_feature (14)..(14): Xaa = Ser or Thr
  misc_feature (18)..(18): Xaa = Arg or Ser
  misc_feature (19)..(19): Xaa = Ala or Val
  misc_feature (20)..(20): Xaa = Ser or Thr
  misc_feature (39)..(39): Xaa = Lys or Arg
  misc_feature (40)..(40): Xaa = Pro or Ser
  misc_feature (41)..(41): Xaa = Gly or Asn
  misc_feature (42)..(42): Xaa = Glu or Gln
  misc_feature (43)..(43): Xaa = Ala or Ser
  misc_feature (60)..(60): Xaa = Ala or Ser
  misc_feature (74)..(74): Xaa = Ser or Thr
  misc_feature (76)..(76): Xaa = Asn or Ser
  misc_feature (77)..(77): Xaa = Arg or Ser
  misc_feature (78)..(78): Xaa = Leu or Val
  misc_feature (80)..(80): Xaa = Pro or Ser
  misc_feature (84)..(84): Xaa = Ala or Ser
  misc_feature (85)..(85): Xaa = Ile or Val
  misc_feature (100)..(100): Xaa = Ala or Gln
  misc_feature (106)..(106): Xaa = Ile or Leu
  misc_feature (107)..(107): Xaa = Lys or Arg
XIVLTQSPATLSXXPGEXXXLSCRASQSVSTSIHWYQQXXXXXPRLLIKYASRSISGIPXRFSGSGSGTDFTLXIXXXEXEDFXXYYCQQSYSSLYTFGXGTKLEXX

SEQ ID NO: 67 - protein, 125 aa, Artificial Sequence
  general formula 1 of VH
  misc_feature (16)..(16): Xaa = Gly or Arg
  misc_feature (19)..(19): Xaa = Arg or Ser
  misc_feature (40)..(40): Xaa = Ala or Thr
  misc_feature (42)..(42): Xaa = Gly or Lys
  misc_feature (73)..(73): Xaa = Asp or Glu
  misc_feature (77)..(77): Xaa = Asn or Ser
  misc_feature (78)..(78): Xaa = Ser or Thr
  misc_feature (84)..(84): Xaa = Asp or Asn
  misc_feature (88)..(88): Xaa = Ala or Ser
  misc_feature (93)..(93): Xaa = Thr or Val
  misc_feature (119)..(119): Xaa = Thr or Val
  misc_feature (120)..(120): Xaa = Leu or Met
EVQLVESGGGLVQPGXSLXLSCAASGFTFNDYNMAWVRQXPXKGLEWVATILFDGSRTYYRDSVKGRFTISRXNAKXXLYLQMXSLRXEDTAXYYCSTESPYYSEGYYQGYFDYWGQGXXVTVSS

SEQ ID NO: 68 - protein, 23 aa, Artificial Sequence
  general formula 2 of L-FR1
  misc_feature (3)..(3): Xaa = Gln or Val
  misc_feature (8)..(8): Xaa = Pro or Gln
  misc_feature (9)..(9): Xaa = Lys or Ser
  misc_feature (10)..(10): Xaa = Phe or Ser
  misc_feature (11)..(11): Xaa = Leu or Met
  misc_feature (13)..(13): Xaa = Ala or Thr
  misc_feature (20)..(20): Xaa = Ser or Thr
  misc_feature (21)..(21): Xaa = Ile or Val
DIXMTQSXXXXSXSVGDRVXXTC

SEQ ID NO: 69 - protein, 15 aa, Artificial Sequence
  general formula 2 of L-FR2
  misc_feature (8)..(8): Xaa = Lys or Gln
  misc_feature (9)..(9): Xaa = Ala or Ser
WFQQKPGXXPKPLIY

SEQ ID NO: 70 - protein, 32 aa, Artificial Sequence
  general formula 2 of L-FR3
  misc_feature (4)..(4): Xaa = Asp or Ser
  misc_feature (7)..(7): Xaa = Ser or Thr
  misc_feature (21)..(21): Xaa = Asn or Ser
  misc_feature (22)..(22): Xaa = Leu or Val
  misc_feature (24)..(24): Xaa = Pro or Ser
  misc_feature (27)..(27): Xaa = Phe or Leu
  misc_feature (29)..(29): Xaa = Glu or Thr
GVPXRFXGSGSGTDFTLTISXXQXEDXAXYFC

SEQ ID NO: 71 - protein, 10 aa, Artificial Sequence
  general formula 2 of L-FR4
  misc_feature (3)..(3): Xaa = Ala or Gly
  misc_feature (7)..(7): Xaa = Leu or Val
  misc_feature (9)..(9): Xaa = Ile or Leu
  misc_feature (10)..(10): Xaa = Lys or Asn
FGXGTKXEXX

SEQ ID NO: 72 - protein, 25 aa, Artificial Sequence
  general formula 2 of H-FR1
  misc_feature (1)..(1): Xaa = Asp or Gln
  misc_feature (17)..(17): Xaa = Ser or Thr
  misc_feature (25)..(25): Xaa = Ser or Thr
XVQLQESGPGLVKPSQXLSLTCTVX

SEQ ID NO: 73 - protein, 19 aa, Artificial Sequence
  general formula 2 of H-FR2
  misc_feature (8)..(8): Xaa = Phe or Pro
  misc_feature (11)..(11): Xaa = Lys or Asn
  misc_feature (12)..(12): Xaa = Gly or Lys
  misc_feature (16)..(16): Xaa = Ile or Met
AWNWIRQXPGXXLEWXGYI

SEQ ID NO: 74 - protein, 41 aa, Artificial Sequence
  general formula 2 of H-FR3
  misc_feature (11)..(11): Xaa = Ile or Val
  misc_feature (12)..(12): Xaa = Ser or Thr
  misc_feature (14)..(14): Xaa = Ser or Thr
  misc_feature (16)..(16): Xaa = Asp or Asn
  misc_feature (19)..(19): Xaa = Lys or Thr
  misc_feature (23)..(23): Xaa = Phe or Ser
  misc_feature (25)..(25): Xaa = Lys or Gln
  misc_feature (27)..(27): Xaa = Asn or Ser
  misc_feature (31)..(31): Xaa = Ala or Thr
  misc_feature (32)..(32): Xaa = Ala or Glu
  misc_feature (36)..(36): Xaa = Thr or Val
  misc_feature (38)..(38): Xaa = Phe or Tyr
TSYNPSLKSRXXIXRXTSXNQFXLXLXSVTXXDTAXYXCAR

SEQ ID NO: 75 - protein, 11 aa, Artificial Sequence
  general formula 2 of H-FR4
  misc_feature (6)..(6): Xaa = Leu or Thr
  misc_feature (7)..(7): Xaa = Leu or Val
WGQGTXXTVSS

SEQ ID NO: 76 - protein, 107 aa, Artificial Sequence
  general formula 2 of VL
  misc_feature (3)..(3): Xaa = Gln or Val
  misc_feature (8)..(8): Xaa = Pro or Gln
  misc_feature (9)..(9): Xaa = Lys or Ser
  misc_feature (10)..(10): Xaa = Phe or Ser
  misc_feature (11)..(11): Xaa = Leu or Met
  misc_feature (13)..(13): Xaa = Ala or Thr
  misc_feature (20)..(20): Xaa = Ser or Thr
  misc_feature (21)..(21): Xaa = Ile or Val
  misc_feature (42)..(42): Xaa = Lys or Gln
  misc_feature (43)..(43): Xaa = Ala or Ser
  misc_feature (60)..(60): Xaa = Asp or Ser
  misc_feature (63)..(63): Xaa = Ser or Thr
  misc_feature (77)..(77): Xaa = Asn or Ser
  misc_feature (78)..(78): Xaa = Leu or Val
  misc_feature (80)..(80): Xaa = Pro or Ser
  misc_feature (83)..(83): Xaa = Phe or Leu
  misc_feature (85)..(85): Xaa = Glu or Thr
  misc_feature (100)..(100): Xaa = Ala or Gly
  misc_feature (104)..(104): Xaa = Leu or Val
  misc_feature (106)..(106): Xaa = Ile or Leu
  misc_feature (107)..(107): Xaa = Lys or Asn
DIXMTQSXXXXSXSVGDRVXXTCKASQNVGSNVAWFQQKPGXXPKPLIYSASYRYSGVPXRFXGSGSGTDFTLTISXXQXEDXAXYFCHQYNTYPLTFGXGTKXEXX

SEQ ID NO: 77 - protein, 114 aa, Artificial Sequence
  general formula 2 of VH
  misc_feature (1)..(1): Xaa = Asp or Gln
  misc_feature (17)..(17): Xaa = Ser or Thr
  misc_feature (25)..(25): Xaa = Ser or Thr
  misc_feature (41)..(41): Xaa = Phe or Pro
  misc_feature (44)..(44): Xaa = Lys or Asn
  misc_feature (45)..(45): Xaa = Gly or Lys
  misc_feature (49)..(49): Xaa = Ile or Met
  misc_feature (68)..(68): Xaa = Ile or Val
  misc_feature (69)..(69): Xaa = Ser or Thr
  misc_feature (71)..(71): Xaa = Ser or Thr
  misc_feature (73)..(73): Xaa = Asp or Asn
  misc_feature (76)..(76): Xaa = Lys or Thr
  misc_feature (80)..(80): Xaa = Phe or Ser
  misc_feature (82)..(82): Xaa = Lys or Gln
  misc_feature (84)..(84): Xaa = Asn or Ser
  misc_feature (88)..(88): Xaa = Ala or Thr
  misc_feature (89)..(89): Xaa = Ala or Glu
  misc_feature (93)..(93): Xaa = Thr or Val
  misc_feature (95)..(95): Xaa = Phe or Tyr
  misc_feature (109)..(109): Xaa = Leu or Thr
  misc_feature (110)..(110): Xaa = Leu or Val
XVQLQESGPGLVKPSQXLSLTCTVXGYSITSDYAWNWIRQXPGXXLEWXGYISYSGRTSYNPSLKSRXXIXRXTSXNQFXLXLXSVTXXDTAXYXCARYWGDYWGQGTXXTVSS